European Patent Application EP 4 591 878 A2, published July 30, 2025. Title: Antibody Binding to Tie2 and Use Thereof. Applicant: Institute for Basic Science. Application EP. The sequence listing filed with the application follows.

SEQUENCE LISTING (78 sequences)

SEQ ID NO: 1 - protein, 1124 aa, synthetic construct
MDSLASLVLCGVSLLLSGTVEGAMDLILINSLPLVSDAETSLTCIASGWRPHEPITIGRDFEALMNQHQDPLEVTQDVTREWAKKVVWKREKASKINGAYFCEGRVRGEAIRIRTMKMRQQASFLPATLTMTVDKGDNVNISFKKVLIKEEDAVIYKNGSFIHSVPRHEVPDILEVHLPHAQPQDAGVYSARYIGGNLFTSAFTRLIVRRCEAQKWGPECNHLCTACMNNGVCHEDTGECICPPGFMGRTCEKACELHTFGRTCKERCSGQEGCKSYVFCLPDPYGCSCATGWKGLQCNEACHPGFYGPDCKLRCSCNNGEMCDRFQGCLCSPGWQGLQCEREGIQRMTPKIVDLPDHIEVNSGKFNPICKASGWPLPTNEEMTLVKPDGTVLHPKDFNHTDHFSVAIFTIHRILPPDSGVWVCSVNTVAGMVEKPFNISVKVLPKPLNAPNVIDTGHNFAVINISSEPYFGDGPIKSKKLLYKPVNHYEAWQHIQVTNEIVTLNYLEPRTEYELCVQLVRRGEGGEGHPGPVRRFTTASIGLPPPRGLNLLPKSQTTLNLTWQPIFPSSEDDFYVEVERRSVQKSDQQNIKVPGNLTSVLLNNLHPREQYVVRARVNTKAQGEWSEDLTAWTLSDILPPQPENIKISNITHSSAVISWTILDGYSISSITIRYKVQGKNEDQHVDVKIKNATITQYQLKGLEPETAYQVDIFAENNIGSSNPAFSHELVTLPESQAPADLGGGKMLLIAILGSAGMTCLTVLLAFLIILQLKRANVQRRMAQAFQNVREEPAVQFNSGTLALNRKVKNNPDPTIYPVLDWNDIKFQDVIGEGNFGQVLKARIKKDGLRMDAAIKRMKEYASKDDHRDFAGELEVLCKLGHHPNIINLLGACEHRGYLYLAIEYAPHGNLLDFLRKSRVLETDPAFAIANSTASTLSSQQLLHFAADVARGMDYLSQKQFIHRDLAARNILVGENYVAKIADFGLSRGQEVYVKKTMGRLPVRWMAIESLNYSVYTTNSDVWSYGVLLWEIVSLGGTPYCGMTCAELYEKLPQGYRLEKPLNCDDEVYDLMRQCWREKPYERPSFAQILVSLNRMLEERKTYVNTTLYEKFTYAGIDCSAEEAA

SEQ ID NO: 2 - protein, 390 aa, synthetic construct
TPKIVDLPDHIEVNSGKFNPICKASGWPLPTNEEMTLVKPDGTVLHPKDFNHTDHFSVAIFTIHRILPPDSGVWVCSVNTVAGMVEKPFNISVKVLPKPLNAPNVIDTGHNFAVINISSEPYFGDGPIKSKKLLYKPVNHYEAWQHIQVTNEIVTLNYLEPRTEYELCVQLVRRGEGGEGHPGPVRRFTTASIGLPPPRGLNLLPKSQTTLNLTWQPIFPSSEDDFYVEVERRSVQKSDQQNIKVPGNLTSVLLNNLHPREQYVVRARVNTKAQGEWSEDLTAWTLSDILPPQPENIKISNITHSSAVISWTILDGYSISSITIRYKVQGKNEDQHVDVKIKNATITQYQLKGLEPETAYQVDIFAENNIGSSNPAFSHELVTLPESQAP

SEQ ID NO: 3 - protein, 5 aa, synthetic construct
SYWMN

SEQ ID NO: 4 - protein, 17 aa, synthetic construct
MIHPSDSETRLNQKFKD

SEQ ID NO: 5 - protein, 6 aa, synthetic construct
GNYFDC

SEQ ID NO: 6 - protein, 11 aa, synthetic construct
RASQDIGISLN

SEQ ID NO: 7 - protein, 7 aa, synthetic construct
ATSILDS

SEQ ID NO: 8 - protein, 9 aa, synthetic construct
LQYASSPWT

SEQ ID NO: 9 - protein, 115 aa, synthetic construct
QVQLQQPGAELVRPGASVKLSCKASGYSFTSYWMNWVKQRPGQGLEWIGMIHPSDSETRLNQKFKDKATLTVDKSSSTAYLQLSSPTSEDSAVYYCARGNYFDCWGQGTTLTVSS

SEQ ID NO: 10 - DNA, 345 bp, synthetic construct
  source 1..345: mol_type = other DNA
caggtccaactgcagcagcctggggctgagctggtgaggcctggagcttcagtgaagctgtcctgcaaggcttctggctactccttcaccagctactggatgaactgggtgaagcagaggcctggacaaggccttgagtggattggcatgattcatccttccgatagtgaaactaggttaaatcagaagttcaaggacaaggccacattgactgtagacaaatcctccagcacagcctacttgcaactcagcagcccgacatctgaggactctgcggtctattactgtgcaagggggaactactttgactgctggggccaaggcaccactctcacagtctcctca

SEQ ID NO: 11 - protein, 107 aa, synthetic construct
DIQMTQSPSSLSASLGERVSLTCRASQDIGISLNWLQQEPDGTIKRLIYATSILDSGVPKRFSGSRSGSDYSLTISSLESEDFVDYYCLQYASSPWTFGGGTKLEIK

SEQ ID NO: 12 - DNA, 321 bp, synthetic construct
  source 1..321: mol_type = other DNA
gacatccagatgacccagtctccatcctccttatctgcctctctgggagaaagggtcagtctcacttgtcgggcaagtcaggacattggtattagcttaaactggcttcagcaggaaccagatggaactattaaacgcctgatctacgccacatccattttagattctggtgtccccaaaaggttcagtggcagtaggtctgggtcagattattctctcaccatcagcagccttgagtctgaagattttgtagactattactgtctacaatatgctagttctccgtggacgttcggtggaggcaccaagctggaaatcaaa

SEQ ID NO: 13 - protein, 5 aa, synthetic construct
SYWMN

SEQ ID NO: 14 - protein, 17 aa, synthetic construct
MIHPSDSETRLNQKFKD

SEQ ID NO: 15 - protein, 6 aa, synthetic construct
GYYFGY

SEQ ID NO: 16 - protein, 11 aa, synthetic construct
RASQDIGISLN

SEQ ID NO: 17 - protein, 7 aa, synthetic construct
ATSNLDS

SEQ ID NO: 18 - protein, 9 aa, synthetic construct
LQYASSPPT

SEQ ID NO: 19 - protein, 115 aa, synthetic construct
QVQLQQPGADLVRPGASVKLSCKASGYSFTSYWMNWVKQRPGQGLEWIGMIHPSDSETRLNQKFKDKATLTVDKSSSTAYMQLSSPTSEDSAVYYCAKGYYFGYWGQGTTLTVSS

SEQ ID NO: 20 - DNA, 345 bp, synthetic construct
  source 1..345: mol_type = other DNA
caggtccaactgcagcagcctggggctgacctggtgaggcctggagcttcagtgaagctgtcctgcaaggcttctggctactccttcaccagctactggatgaactgggtgaagcagaggcctggacaaggccttgagtggattggcatgattcatccttccgatagtgaaactaggttaaatcagaagttcaaggacaaggccacattgactgtagacaaatcctccagcacagcctacatgcaactcagcagcccgacatctgaggactctgcggtctattactgtgcaaaggggtactactttggctactggggccaaggcaccactctcacagtctcctca

SEQ ID NO: 21 - protein, 107 aa, synthetic construct
DIQMTQSPSSLSASLGERVSLTCRASQDIGISLNWLQQEPDGTIKRLIYATSNLDSGVPKRFSGSRSGSDYSLTISSLESEDFVDYYCLQYASSPPTFGGGTKLEIK

SEQ ID NO: 22 - DNA, 321 bp, synthetic construct
  source 1..321: mol_type = other DNA
gacatccagatgacccagtctccatcctccttatctgcctctctgggagaaagagtcagtctcacttgtcgggcaagtcaggacattggtattagtttaaactggcttcagcaggaaccagatggaactattaaacgcctgatctacgccacatccaatttagattctggtgtccccaaaaggttcagtggcagtaggtctgggtcagattattctctcaccatcagcagccttgagtctgaagattttgtagactattactgtctacaatatgctagttctcctccgacgttcggtggaggcaccaagctggaaatcaaa

SEQ ID NO: 23 - protein, 5 aa, synthetic construct
SYWMN

SEQ ID NO: 24 - protein, 17 aa, synthetic construct
MIHPSDSETRLNQKFMD

SEQ ID NO: 25 - protein, 6 aa, synthetic construct
GLYGNS

SEQ ID NO: 26 - protein, 11 aa, synthetic construct
RASQDIGISLN

SEQ ID NO: 27 - protein, 7 aa, synthetic construct
ATSSLDS

SEQ ID NO: 28 - protein, 9 aa, synthetic construct
LQYASSPYT

SEQ ID NO: 29 - protein, 115 aa, synthetic construct
QVQLQQPGAELVRPGASVKLSCKASGYSFTSYWMNWVKQRPGQGLEWIGMIHPSDSETRLNQKFMDKATLTVDKSSSTAYMQLSSPTSEDSAVYYCARGLYGNSWGQGTLVTVSA

SEQ ID NO: 30 - DNA, 345 bp, synthetic construct
  source 1..345: mol_type = other DNA
caggtccaactgcagcagcctggggctgagctggtgaggcctggagcttcagtgaagctgtcctgcaaggcttctggctactccttcaccagctactggatgaactgggtgaagcagaggcctggacaaggccttgagtggattggcatgattcatccttccgatagtgaaactaggttaaatcagaagttcatggacaaggccacattgactgtagacaaatcctccagcacagcctacatgcagctcagcagcccgacatctgaggactctgcggtctattactgtgctcgtggcctctatggtaactcttggggccaagggactctggtcactgtctctgca

SEQ ID NO: 31 - protein, 107 aa, synthetic construct
DIQMTQSPSSLSASLGERVSLTCRASQDIGISLNWLQQEPDGTIKRLIYATSSLDSGVPKRFSGSRSGSDYSLTISSLESEDFVDYYCLQYASSPYTFGGGTKLEIK

SEQ ID NO: 32 - DNA, 321 bp, synthetic construct
  source 1..321: mol_type = other DNA
gacatccagatgacccagtctccatcctccttatctgcctctctgggagaaagagtcagtctcacttgtcgggcaagtcaggacattggtattagcttaaactggcttcagcaggaaccagatggaactattaaacgcctgatctacgccacatccagtttagattctggtgtccccaaaaggttcagtggcagtaggtctgggtcagattattctctcaccatcagcagccttgagtctgaagattttgtagactattactgtctacaatatgctagttctccgtacacgttcggaggggggaccaagctggaaataaaa

SEQ ID NO: 33 - protein, 5 aa, synthetic construct
SYWMN

SEQ ID NO: 34 - protein, 17 aa, synthetic construct
MIHPSDSETRLNQKFKD

SEQ ID NO: 35 - protein, 6 aa, synthetic construct
GYYFDY

SEQ ID NO: 36 - protein, 11 aa, synthetic construct
RASQDIGISLN

SEQ ID NO: 37 - protein, 7 aa, synthetic construct
ATSSLDS

SEQ ID NO: 38 - protein, 9 aa, synthetic construct
LQYVSSPWT

SEQ ID NO: 39 - protein, 115 aa, synthetic construct
QVQLQQPGAELVRPGASVKLSCKASGYSFTSYWMNWVKQRPGQGLEWIGMIHPSDSETRLNQKFKDKATLTVDKSSSTAYMQLSSPTSEDSAVYYCARGYYFDYWGQGTTLTVSS

SEQ ID NO: 40 - DNA, 345 bp, synthetic construct
  source 1..345: mol_type = other DNA
caggtccaactgcagcagcctggggctgagctggtgaggcctggagcttcagtgaagctgtcctgcaaggcttctggctactccttcaccagctactggatgaactgggtgaagcagaggcctggacaaggccttgagtggattggcatgattcatccttccgatagtgaaactaggttaaatcagaagttcaaggacaaggccacattgactgtagacaaatcctccagcacagcctacatgcaactcagcagcccgacatctgaggactctgcggtctattactgtgcaagaggctactactttgactactggggccaaggcaccactctcacagtctcctca

SEQ ID NO: 41 - protein, 107 aa, synthetic construct
DIQMTQSPSSLSASLGERVSLTCRASQDIGISLNWLQQEPDGTIKRLIYATSSLDSGVPKRFTGSRSGSDYSLTISSLESEDFVDYYCLQYVSSPWTFGGGTKLEIK

SEQ ID NO: 42 - DNA, 321 bp, synthetic construct
  source 1..321: mol_type = other DNA
gacatccagatgacccagtctccatcctccttatctgcctctctgggagaaagagtcagtctcacttgtcgggcaagtcaggacattggtattagcttaaactggcttcagcaggaaccagatggaactattaaacgcctgatctacgccacatccagtttagattctggtgtccccaagaggttcactggcagtaggtctgggtcagattattctctcaccatcagcagccttgagtctgaagattttgtagactattactgtctacaatatgttagttctccgtggacgttcggtggaggcaccaagctggaaatcaaa

SEQ ID NO: 43 - protein, 5 aa, synthetic construct
SYWMN

SEQ ID NO: 44 - protein, 17 aa, synthetic construct
MIHPSDSETRLNQKFKD

SEQ ID NO: 45 - protein, 7 aa, synthetic construct
LTIYFDY

SEQ ID NO: 46 - protein, 11 aa, synthetic construct
RASQDIGISLN

SEQ ID NO: 47 - protein, 7 aa, synthetic construct
ATSSLDS

SEQ ID NO: 48 - protein, 9 aa, synthetic construct
LQYASSPYT

SEQ ID NO: 49 - protein, 116 aa, synthetic construct
QVQLQQPGADLVRPGASVTLSCKASGYSFTSYWMNWVKQRPGQGLEWIGMIHPSDSETRLNQKFKDKATLTVDKSSSTAYMQLRSPTSEDSAVYYCAGLTIYFDYWGQGTTLTVSS

SEQ ID NO: 50 - DNA, 348 bp, synthetic construct
  source 1..348: mol_type = other DNA
caggtccaactacagcagcctggggctgacctggtgaggcctggagcttcagtgacgctgtcctgcaaggcttctggctactccttcaccagctactggatgaactgggtgaagcagaggcctggacaaggcctggagtggattggcatgattcatccttccgatagtgaaactaggttaaatcagaagttcaaggacaaggccacattgactgtagacaaatcctccagcacagcctacatgcaactccgcagcccgacatctgaggactctgcggtctattactgtgcaggcctaactatttactttgactattggggccaaggcaccactctcacagtctcctca

SEQ ID NO: 51 - protein, 107 aa, synthetic construct; identical to SEQ ID NO: 31

SEQ ID NO: 52 - DNA, 321 bp, synthetic construct; identical to SEQ ID NO: 32
  source 1..321: mol_type = other DNA

SEQ ID NO: 53 - protein, 115 aa, synthetic construct
QVQLVQSGAEVKKPGASVKVSCKASGYTFTSYWMNWVRQAPGQGLEWMGMIHPSDSETRLNQKFMDRVTMTRDTSTSTVYMELSSLRSEDTAVYYCARGLYGNSWGQGTLVTVSS

SEQ ID NO: 54 - protein, 107 aa, synthetic construct
DIQMTQSPSSLSASVGDRVTITCRASQDIGISLNWYQQKPGKAPKRLIYATSSLDSGVPSRFSGSGSGTEFTLTISSLQPEDFATYYCLQYASSPYTFGQGTKVEIK

SEQ ID NO: 55 - DNA, 345 bp, synthetic construct
  source 1..345: mol_type = other DNA
caggtgcagctggtccaatccggggctgaggtgaagaagcctggagcatcagtgaaagtttcatgcaaagctagtggttacaccttcaccagctattggatgaactgggtgcggcaggcccccggtcaggggcttgagtggatgggcatgatccacccatccgactctgagactaggctgaaccagaagtttatggatagagtgaccatgacaagagatacgtccacttctactgtctatatggaactgagcagtctgagatctgaagacacagccgtttactactgtgctcgcggactctatggcaatagctggggccaaggaacattggtaaccgtctcttct

SEQ ID NO: 56 - DNA, 321 bp, synthetic construct
  source 1..321: mol_type = other DNA
gacatccagatgacccaatctccctcctccctgagcgcatccgtgggggatagagtgaccataacctgccgggcctctcaggacatcggtatttctttgaattggtatcagcagaagcccgggaaggcccctaaacgcctgatctatgctacttccagtctggacagcggggtcccgtcaaggttttcaggcagtggatcaggcacagagtttacactcacaatttcgagcctgcagcctgaagatttcgccacttattactgtcttcaatacgctagctctccatacacgttcggccagggaaccaaggttgagattaaa

SEQ ID NO: 57 - protein, 115 aa, synthetic construct; identical to SEQ ID NO: 53

SEQ ID NO: 58 - protein, 107 aa, synthetic construct
DIQMTQSPSSLSASVGDRVTITCRASQDIGISLNWLQQEPGKAPKRLIYATSSLDSGVPKRFSGSGSGTEFTLTISSLQPEDFATYYCLQYASSPYTFGQGTKVEIK

SEQ ID NO: 59 - DNA, 345 bp, synthetic construct; identical to SEQ ID NO: 55
  source 1..345: mol_type = other DNA

SEQ ID NO: 60 - DNA, 321 bp, synthetic construct
  source 1..321: mol_type = other DNA
gacatccagatgactcagtccccctcgagcctctcagcttctgttggagacagagtgacaattacatgccgggcctcacaggatattgggatctccctgaactggctgcaacaggaaccaggaaaggcccctaagcgcctgatatatgccacatcctctcttgactcaggggtcccaaagaggtttagcggcagtggatcaggtactgagttcactctcaccatctctagcctgcagcctgaggattttgcaacctactattgtttgcaatacgctagttccccctacacgttcggccagggcaccaaagtggaaatcaaa

SEQ ID NO: 61 - protein, 115 aa, synthetic construct
QVQLVQSGAEVKKPGASVKVSCKASGYTFTSYWMNWVRQRPGQGLEWIGMIHPSDSETRLNQKFMDRVTMTRDTSTSTVYMELSSLRSEDTAVYYCARGLYGNSWGQGTLVTVSS

SEQ ID NO: 62 - protein, 107 aa, synthetic construct; identical to SEQ ID NO: 54

SEQ ID NO: 63 - DNA, 345 bp, synthetic construct
  source 1..345: mol_type = other DNA
caagtccagctcgtgcagtctggcgctgaggtgaaaaagcccggggcctcagtgaaggtttcttgcaaggcaagcggctacacctttacctcctattggatgaattgggtgcgacagcggccaggccaggggttggagtggatcggaatgattcaccctagtgactcagaaactaggctgaaccagaaattcatggacagagtcacaatgacgcgcgatacaagcactagtacagtttacatggagctgagcagcctgagatcggaagatactgccgtgtattactgtgctaggggactgtatggaaactcttggggtcaaggcacccttgtaaccgtctcctcc

SEQ ID NO: 64 - DNA, 321 bp, synthetic construct; identical to SEQ ID NO: 56
  source 1..321: mol_type = other DNA

SEQ ID NO: 65 - protein, 115 aa, synthetic construct; identical to SEQ ID NO: 61

SEQ ID NO: 66 - protein, 107 aa, synthetic construct; identical to SEQ ID NO: 58

SEQ ID NO: 67 - DNA, 345 bp, synthetic construct; identical to SEQ ID NO: 63
  source 1..345: mol_type = other DNA

SEQ ID NO: 68 - DNA, 321 bp, synthetic construct; identical to SEQ ID NO: 60
  source 1..321: mol_type = other DNA

SEQ ID NO: 69 - protein, 156 aa, synthetic construct
VQKSDQQNIKVPGNLTSVLLNNLHPREQYVVRARVNTKAQGEWSEDLTAWTLSDILPPQPENIKISNITHSSAVISWTILDGYSISSITIRYKVQGKNEDQHVDVKIKNATITQYQLKGLEPETAYQVDIFAENNIGSSNPAFSHELVTLPESQAP

SEQ ID NO: 70 - protein, 13 aa, synthetic construct
WTLSDILPPQPEN

SEQ ID NO: 71 - protein, 10 aa, synthetic construct
SDILPPQPEN

SEQ ID NO: 72 - protein, 7 aa, synthetic construct
VISWTIL

SEQ ID NO: 73 - protein, 17 aa, synthetic construct
IFAENNIGSSNPAFSHE

SEQ ID NO: 74 - protein, 16 aa, synthetic construct
FAENNIGSSNPAFSHE

SEQ ID NO: 75 - protein, 15 aa, synthetic construct
AENNIGSSNPAFSHE

SEQ ID NO: 76 - protein, 8 aa, synthetic construct
SHELVTLP

SEQ ID NO: 77 - protein, 12 aa, synthetic construct
TLSDILPPQPEN

SEQ ID NO: 78 - protein, 14 aa, synthetic construct
FAENNIGSSNPAFS